European Patent Specification EP 3 634 997 B1, published February 26, 2025. Title: NOVEL ANTI-HSA ANTIBODIES. Applicant: Numab Innovation AG. The sequence listing filed with the application follows.

SEQUENCE LISTING (10 sequences)

SEQ ID NO: 1 - protein, 112 aa, Artificial Sequence
  recombinant antibody sequence
DIQMTQSPSSLSASVGDRVTITCQSSESVYSNNQLSWYQQKPGQPPKLLIYDASDLASGVPSRFSGSGSGTDFTLTISSLQPEDFATYYCAGGFSSSSDTAFGGGTKLTVLG

SEQ ID NO: 2 - protein, 121 aa, Artificial Sequence
  recombinant antibody sequence
EVQLVESGGGLVQPGGSLRLSCAASGFSLSSNAMGWVRQAPGKGLEYIGIISVGGFTYYASWAKGRFTISRDNSKNTVYLQMNSLRAEDTATYFCARDRHGGDSSGAFYLWGQGTLVTVSS

SEQ ID NO: 3 - protein, 110 aa, Artificial Sequence
  recombinant antibody sequence
DVVMTQSPSSLSASVGDRVTITCQASQIISSRSAWYQQKPGQPPKLLIYQASKLASGVPSRFSGSGSGTDFTLTISSLQPEDFATYYCQCTYIDSNFGAFGGGTKLTVLG

SEQ ID NO: 4 - protein, 121 aa, Artificial Sequence
  recombinant antibody sequence
EVQLVESGGGLVQPGGSLRLSCAASGFSFSSSYWICWVRQAPGKGLEWVGCVFTGDGTTYYASWAKGRFTISRDNSKNTVYLQMNSLRAEDTATYFCARPVSVYYYGMDLWGQGTLVTVSS

SEQ ID NO: 5 - protein, 20 aa, Artificial Sequence
  recombinant antibody sequence
GGGGSGGGGSGGGGSGGGGS

SEQ ID NO: 6 - protein, 11 aa, Artificial Sequence
  recombinant antibody sequence
FGTGTKVTVLG

SEQ ID NO: 7 - protein, 11 aa, Artificial Sequence
  recombinant antibody sequence
FGGGTKLTVLG

SEQ ID NO: 8 - protein, 11 aa, Artificial Sequence
  recombinant antibody sequence
WGQGTLVTVSS

SEQ ID NO: 9 - protein, 5 aa, Artificial Sequence
  recombinant antibody sequence
GGGGS

SEQ ID NO: 10 - protein, 15 aa, Artificial Sequence
  recombinant antibody sequence
GGGGSGGGGSGGGGS